European Patent Application EP 4 219 534 A2, published August 2, 2023. The sequence listing filed with the application follows.

SEQUENCE LISTING (2 sequences)

SEQ ID NO: 1 - protein, 60 aa, Homo sapiens
KAVLTIDEKGTEAAGAMFLEAIPMSIPPEVKFNKPFVFLMIEQNTKSPLFMGKVVNPTQK

SEQ ID NO: 2 - protein, 30 aa, Homo sapiens
  misc_feature (2)..(2): Xaa can be any naturally occurring amino acid
MXIPPEVKFNKPFVFLMIDQNTKVPLFMGK